European Patent Specification EP 4 196 792 B1, published July 1, 2026. Title: BICYCLE CONJUGATES SPECIFIC FOR NECTIN-4 AND USES THEREOF. Applicant: BicycleTx Limited. The sequence listing filed with the application follows.

SEQUENCE LISTING (1 sequence)

SEQ ID NO: 1 - protein, 17 aa, Artificial
  Synthetic Peptide
  Xaa (1)..(1): Xaa is B-Ala
  Xaa (2)..(2): Xaa is Sar10
  Xaa (5)..(5): Xaa is 1Nal
  Xaa (9)..(9): Xaa is HArg
  Xaa (15)..(15): Xaa is HyP
XXCPXDCMXDWSTPXWC